European Patent Application EP 4 523 704 A1, published March 19, 2025. Title: 喜树碱类衍生物及配体-药物偶联物. Applicant: 先声再明医药有限公司. Application CN. The sequence listing filed with the application follows.

SEQUENCE LISTING (105 sequences)

SEQ ID NO: 1 - protein, 120 aa, Artificial Sequence [sequence omitted]

SEQ ID NO: 2 - protein, 107 aa, Artificial Sequence [sequence omitted]

SEQ ID NO: 3 - protein, 119 aa, Artificial Sequence [sequence omitted]

SEQ ID NO: 4 - protein, 107 aa, Artificial Sequence [sequence omitted]

SEQ ID NO: 5 - protein, 330 aa, Artificial Sequence
ASTKGPSVFPLAPSSKSTSGGTAALGCLVKDYFPEPVTVSWNSGALTSGVHTFPAVLQSSGLYSLSSVVTVPSSSLGTQTYICNVNHKPSNTKVDKKVEPKSCDKTHTCPPCPAPELLGGPSVFLFPPKPKDTLMISRTPEVTCVVVDVSHEDPEVKFNWYVDGVEVHNAKTKPREEQYNSTYRVVSVLTVLHQDWLNGKEYKCKVSNKALPAPIEKTISKAKGQPREPQVYTLPPSREEMTKNQVSLTCLVKGFYPSDIAVEWESNGQPENNYKTTPPVLDSDGSFFLYSKLTVDKSRWQQGNVFSCSVMHEALHNHYTQKSLSLSPGK

SEQ ID NO: 6 - protein, 107 aa, Artificial Sequence [sequence omitted]

SEQ ID NO: 7 - protein, 5 aa, Artificial Sequence
DTYIH

SEQ ID NO: 8 - protein, 17 aa, Artificial Sequence
RIYPTNGYTRYADSVKG

SEQ ID NO: 9 - protein, 11 aa, Artificial Sequence
WGGDGFYAMDY

SEQ ID NO: 10 - protein, 11 aa, Artificial Sequence
RASQDVNTAVA

SEQ ID NO: 11 - protein, 7 aa, Artificial Sequence
SASFLYS

SEQ ID NO: 12 - protein, 9 aa, Artificial Sequence
QQHYTTPPT

SEQ ID NO: 13 - protein, 5 aa, Artificial Sequence
DYTMD

SEQ ID NO: 14 - protein, 17 aa, Artificial Sequence
DVNPNSGGSIYNQRFKG

SEQ ID NO: 15 - protein, 10 aa, Artificial Sequence
NLGPSFYFDY

SEQ ID NO: 16 - protein, 11 aa, Artificial Sequence
KASQDVSIGVA

SEQ ID NO: 17 - protein, 7 aa, Artificial Sequence
SASYRYT

SEQ ID NO: 18 - protein, 9 aa, Artificial Sequence
QQYYIYPYT

SEQ ID NO: 19 - protein, 124 aa, Artificial Sequence
EVTLRESGPALVKPTQTLTLTCTFSGFSLYTSGMGVSWIRQPPGKALEWLANIYWDNDKRYNPSLKSRLTISKDTSGNQVVLTMTNMDPVDTATYYCARSFLYYGNSHWYFDVWGQGTTVTVSS

SEQ ID NO: 20 - protein, 106 aa, Artificial Sequence
EIVLTQSPATLSLSPGERATLSCSASSSVSYMYWYQQKPGQAPRLLIYRTSNLASGIPARFSGSGSGTDFTLTISSLEPEDFAVYYCQQYHSYPPTFGQGTKLEIK

SEQ ID NO: 21 - protein, 121 aa, Artificial Sequence
EVTLKESGPALVKPTQTLTLTCTFSGFSLSTFGLGVGWIRQPPGKALEWLAHIWWDTAKNFNPVLKSRLTVSKDTSKNQVVLTMTNMDPVDTATYYCVRIGNYGSPYFDYWGQGTTVTVSS

SEQ ID NO: 22 - protein, 107 aa, Artificial Sequence
LIQMTQSPSSLSASVGDRVTITCLASQSIGTYLAWYQQKPGKAPKLLIYAATSLTDGVPSRFSGSGSGTDFTLTISSLQPEDFATYYCQQVHSSPYSFGGGTKVEIK

SEQ ID NO: 23 - protein, 7 aa, Artificial Sequence
TSGMGVS

SEQ ID NO: 24 - protein, 16 aa, Artificial Sequence
NIYWDNDKRYNPSLKS

SEQ ID NO: 25 - protein, 14 aa, Artificial Sequence
SFLYYGNSHWYFDV

SEQ ID NO: 26 - protein, 10 aa, Artificial Sequence
SASSSVSYMY

SEQ ID NO: 27 - protein, 7 aa, Artificial Sequence
RTSNLAS

SEQ ID NO: 28 - protein, 9 aa, Artificial Sequence
QQYHSYPPT

SEQ ID NO: 29 - protein, 7 aa, Artificial Sequence
TFGLGVG

SEQ ID NO: 30 - protein, 16 aa, Artificial Sequence
HIWWDTAKNFNPVLKS

SEQ ID NO: 31 - protein, 11 aa, Artificial Sequence
IGNYGSPYFDY

SEQ ID NO: 32 - protein, 11 aa, Artificial Sequence
LASQSIGTYLA

SEQ ID NO: 33 - protein, 7 aa, Artificial Sequence
AATSLTD

SEQ ID NO: 34 - protein, 9 aa, Artificial Sequence
QQVHSSPYS

SEQ ID NO: 35 - protein, 585 aa, Artificial Sequence
EVQLVESGGGLVQPGGSLRLSCAASGFTFTDYTMDWVRQAPGKGLEWVADVNPNSGGSIYNQRFKGRFTLSVDRSKNTLYLQMNSLRAEDTAVYYCARNLGPSFYFDYWGQGTLVTVSSGGGGSGGGGSGGGGSEVTLKESGPALVKPTQTLTLTCTFSGFSLSTFGLGVGWIRQPPGKALEWLAHIWWDTAKNFNPVLKSRLTVSKDTSKNQVVLTMTNMDPVDTATYYCVRIGNYGSPYFDYWGQGTTVTVSSASTKGPSVFPLAPSSKSTSGGTAALGCLVKDYFPEPVTVSWNSGALTSGVHTFPAVLQSSGLYSLSSVVTVPSSSLGTQTYICNVNHKPSNTKVDKKVEPKSCDKTHTCPPCPAPELLGGPSVFLFPPKPKDTLMISRTPEVTCVVVDVSHEDPEVKFNWYVDGVEVHNAKTKPREEQYNSTYRVVSVLTVLHQDWLNGKEYKCKVSNKALPAPIEKTISKAKGQPREPQVYTLPPSREEMTKNQVSLTCLVKGFYPSDIAVEWESNGQPENNYKTTPPVLDSDGSFFLYSKLTVDKSRWQQGNVFSCSVMHEALHNHYTQKSLSLSPGK

SEQ ID NO: 36 - protein, 336 aa, Artificial Sequence
DIQMTQSPSSLSASVGDRVTITCKASQDVSIGVAWYQQKPGKAPKLLIYSASYRYTGVPSRFSGSGSGTDFTLTISSLQPEDFATYYCQQYYIYPYTFGQGTKVEIKGGGGSGGGGSGGGGSLIQMTQSPSSLSASVGDRVTITCLASQSIGTYLAWYQQKPGKAPKLLIYAATSLTDGVPSRFSGSGSGTDFTLTISSLQPEDFATYYCQQVHSSPYSFGGGTKVEIKRTVAAPSVFIFPPSDEQLKSGTASVVCLLNNFYPREAKVQWKVDNALQSGNSQESVTEQDSKDSTYSLSSTLTLSKADYEKHKVYACEVTHQGLSSPVTKSFNRGEC

SEQ ID NO: 37 - protein, 122 aa, Artificial Sequence
EVQLVQSGAEVKKPGASVKVSCKASGYTFTRNFMHWVRQAPGQGLEWMGWIYPGDGETEYAQKFQGRVTITADTSTSTAYMELSSLRSEDTAVYYCARGVYGGFAGGYFDFWGQGTLVTVSS

SEQ ID NO: 38 - protein, 106 aa, Artificial Sequence
DIQMTQSPSSLSASVGDRVTITCKASQNIYKNLAWYQQKPGKAPKLLIYDANTLQTGVPSRFSGSGSGSDFTLTISSLQPEDFATYFCQQYYSGWAFGQGTKVEIK

SEQ ID NO: 39 - protein, 330 aa, Artificial Sequence
ASTKGPSVFPLAPSSKSTSGGTAALGCLVKDYFPEPVTVSWNSGALTSGVHTFPAVLQSSGLYSLSSVVTVPSSSLGTQTYICNVNHKPSNTKVDKRVEPKSCDKTHTCPPCPAPELLGGPSVFLFPPKPKDTLMISRTPEVTCVVVDVSHEDPEVKFNWYVDGVEVHNAKTKPREEQYNSTYRVVSVLTVLHQDWLNGKEYKCKVSNKALPAPIEKTISKAKGQPREPQVYTLPPSREEMTKNQVSLTCLVKGFYPSDIAVEWESNGQPENNYKTTPPVLDSDGSFFLYSKLTVDKSRWQQGNVFSCSVMHEALHNHYTQKSLSLSPGK

SEQ ID NO: 40 - protein, 5 aa, Artificial Sequence
RNFMH

SEQ ID NO: 41 - protein, 17 aa, Artificial Sequence
WIYPGDGETEYAQKFQG

SEQ ID NO: 42 - protein, 13 aa, Artificial Sequence
GVYGGFAGGYFDF

SEQ ID NO: 43 - protein, 11 aa, Artificial Sequence
KASQNIYKNLA

SEQ ID NO: 44 - protein, 7 aa, Artificial Sequence
DANTLQT

SEQ ID NO: 45 - protein, 8 aa, Artificial Sequence
QQYYSGWA

SEQ ID NO: 46 - protein, 118 aa, Artificial Sequence
QVQLLESGGGLVQPGGSLRLSCAASGFTFSSHGMHWVRQAPGKGLEWVSVISGSGSNTGYADSVKGRFTISRDNSKNTLYLQMNSLRAEDTAVYYCARQWGSYAFDSWGQGTLVTVSS

SEQ ID NO: 47 - protein, 108 aa, Artificial Sequence
DIQMTQSPSSLSASVGDRVTITCRASQSISSYLNWYQQKPGKAPKLLIYAVSTLQSGVPSRFSGSGSGTDFTLTISSLQPEDFATYYCQQSGTFPPTTFGQGTKVEIK

SEQ ID NO: 48 - protein, 5 aa, Artificial Sequence
SHGMH

SEQ ID NO: 49 - protein, 17 aa, Artificial Sequence
VISGSGSNTGYADSVKG

SEQ ID NO: 50 - protein, 9 aa, Artificial Sequence
QWGSYAFDS

SEQ ID NO: 51 - protein, 11 aa, Artificial Sequence
RASQSISSYLN

SEQ ID NO: 52 - protein, 7 aa, Artificial Sequence
AVSTLQS

SEQ ID NO: 53 - protein, 10 aa, Artificial Sequence
QQSGTFPPTT

SEQ ID NO: 54 - protein, 117 aa, Artificial Sequence
EVQLVQSGAEVKKPGASVKVSCKASGYTFTDNYINWVRQAPGQRLEWMGWIYPGTGNSYYNEKFKGRVTITVDTSASTAYMELSSLRSEDTAVYLCASSYGDSFDYWGQGTTVTVSS

SEQ ID NO: 55 - protein, 107 aa, Artificial Sequence
DIVMTQSPDSLAVSLGERATINCRASQDIRNYLNWYQQKPGQTPKLLISYTSRLHSGVPDRFSGSGSGTDFTLTISSLQAEDVAVYYCQQYSQLPWTFGGGTKVEIK

SEQ ID NO: 56 - protein, 123 aa, Artificial Sequence
EVQLVQSGAEVKKPGASVKVSCKASGYTFTDYYMAWVRQAPGQGLEWMGYIFPNSGGTDYSQKFKGRVTLTVDKSTSTVYMELSSLRSEDTAVYYCARELGADYGDYYAMDHWGQGTTVTVSS

SEQ ID NO: 57 - protein, 107 aa, Artificial Sequence
DIQMTQSPSSLSASVGDRVTITCRASENIDSYLAWYQQKPGKSPKLLVYSATLLADGVPSRFSGSGSGTDYTLTISSLQPEDFATYYCQHYYRTPPTFGQGTKLEIK

SEQ ID NO: 58 - protein, 5 aa, Artificial Sequence
DNYIN

SEQ ID NO: 59 - protein, 17 aa, Artificial Sequence
WIYPGTGNSYYNEKFKG

SEQ ID NO: 60 - protein, 8 aa, Artificial Sequence
SYGDSFDY

SEQ ID NO: 61 - protein, 11 aa, Artificial Sequence
RASQDIRNYLN

SEQ ID NO: 62 - protein, 7 aa, Artificial Sequence
YTSRLHS

SEQ ID NO: 63 - protein, 9 aa, Artificial Sequence
QQYSQLPWT

SEQ ID NO: 64 - protein, 5 aa, Artificial Sequence
DYYMA

SEQ ID NO: 65 - protein, 17 aa, Artificial Sequence
YIFPNSGGTDYSQKFKG

SEQ ID NO: 66 - protein, 14 aa, Artificial Sequence
ELGADYGDYYAMDH

SEQ ID NO: 67 - protein, 11 aa, Artificial Sequence
RASENIDSYLA

SEQ ID NO: 68 - protein, 7 aa, Artificial Sequence
SATLLAD

SEQ ID NO: 69 - protein, 9 aa, Artificial Sequence
QHYYRTPPT

SEQ ID NO: 70 - protein, 19 aa, Artificial Sequence
MGWSWILLFLLSVTAGVHS

SEQ ID NO: 71 - protein, 120 aa, Artificial Sequence
QVQLVQSGAEVKKPGASVKVSCKASGLTIEDYYMHWVRQAPGQGLEWMGWIDPENGDTEYGPKFQGRVTMTRDTSINTAYMELSRLRSDDTAVYYCAVHNAHYGTWFAYWGQGTLVTVSS

SEQ ID NO: 72 - protein, 113 aa, Artificial Sequence
DVVMTQSPLSLPVTLGQPASISCRSSQSLLHSSGNTYLEWYQQRPGQSPRPLIYKISTRFSGVPDRFSGSGSGTDFTLKISRVEAEDVGVYYCFQGSHVPYTFGGGTKVEIKR

SEQ ID NO: 73 - protein, 330 aa, Artificial Sequence [sequence omitted]

SEQ ID NO: 74 - protein, 5 aa, Artificial Sequence
DYYMH

SEQ ID NO: 75 - protein, 17 aa, Artificial Sequence
WIDPENGDTEYGPKFQG

SEQ ID NO: 76 - protein, 11 aa, Artificial Sequence
HNAHYGTWFAY

SEQ ID NO: 77 - protein, 16 aa, Artificial Sequence
RSSQSLLHSSGNTYLE

SEQ ID NO: 78 - protein, 7 aa, Artificial Sequence
KISTRFS

SEQ ID NO: 79 - protein, 9 aa, Artificial Sequence
FQGSHVPYT

SEQ ID NO: 80 - protein, 116 aa, Artificial Sequence
QVQLQESGPGLVKPSQTLSLTCTVSGYAFTAYNIHWVRQAPGQGLEWMGSFDPYDGGSSYNQKFKDRLTISKDTSKNQVVLTMTNMDPVDTATYYCARGWYYFDYWGHGTLVTVSS

SEQ ID NO: 81 - protein, 107 aa, Artificial Sequence
DIVMTQTPLSLPVTPGEPASISCRASKSISKYLAWYQQKPGQAPRLLIYSGSTLQSGIPPRFSGSGYGTDFTLTINNIESEDAAYYFCQQHDESPYTFGEGTKVEIK

SEQ ID NO: 82 - protein, 127 aa, Artificial Sequence
EVQLLESGGGLVQPGGSLRLSCAASGFTFSNYAMSWVRQAPGKGLEWVSSISHNSGSTYYADSVKGRFTISRDNSKNTLYLQMNSLRAEDTAVYYCAKFISARKSLGRSYSNGMDVWGQGTLVTVSS

SEQ ID NO: 83 - protein, 110 aa, Artificial Sequence
QSVLTQPPSASGTPGQRVTISCTGSSSNIGSNDVTWYQQLPGTAPKLLIYADSKRPSGVPDRFSGSKSGTSASLAISGLRSEDEADYYCGTWDYSLSGYVFGGGTKLTVL

SEQ ID NO: 84 - protein, 117 aa, Artificial Sequence
QVQLRESGPGLVKPSETLSLTCTVSGFDISSYYMSWVRQPPGKGLEWIGAIGISGNAYYASWAKSRVTISRDTSKNQFSLKLSSVTAADTAVYYCARDHPTYGMDLWGPGTLVTVSS

SEQ ID NO: 85 - protein, 106 aa, Artificial Sequence
SYELTQPPSVSVAPGKTARITCEGNNIGSKAVHWYQQKPGQAPVLVIYDDDERPSGIPERFSGSNSGNTATLTISRVEAGDEADYYCQVWDSSAYVFGGGTKLTVL

SEQ ID NO: 86 - protein, 5 aa, Artificial Sequence
AYNIH

SEQ ID NO: 87 - protein, 17 aa, Artificial Sequence
SFDPYDGGSSYNQKFKD

SEQ ID NO: 88 - protein, 7 aa, Artificial Sequence
GWYYFDY

SEQ ID NO: 89 - protein, 11 aa, Artificial Sequence
RASKSISKYLA

SEQ ID NO: 90 - protein, 7 aa, Artificial Sequence
SGSTLQS

SEQ ID NO: 91 - protein, 9 aa, Artificial Sequence
QQHDESPYT

SEQ ID NO: 92 - protein, 5 aa, Artificial Sequence
NYAMS

SEQ ID NO: 93 - protein, 17 aa, Artificial Sequence
SISHNSGSTYYADSVKG

SEQ ID NO: 94 - protein, 18 aa, Artificial Sequence
FISARKSLGRSYSNGMDV

SEQ ID NO: 95 - protein, 13 aa, Artificial Sequence
TGSSSNIGSNDVT

SEQ ID NO: 96 - protein, 7 aa, Artificial Sequence
ADSKRPS

SEQ ID NO: 97 - protein, 11 aa, Artificial Sequence
GTWDYSLSGYV

SEQ ID NO: 98 - protein, 5 aa, Artificial Sequence
SYYMS

SEQ ID NO: 99 - protein, 16 aa, Artificial Sequence
AIGISGNAYYASWAKS

SEQ ID NO: 100 - protein, 9 aa, Artificial Sequence
DHPTYGMDL

SEQ ID NO: 101 - protein, 11 aa, Artificial Sequence
EGNNIGSKAVH

SEQ ID NO: 102 - protein, 7 aa, Artificial Sequence
DDDERPS

SEQ ID NO: 103 - protein, 9 aa, Artificial Sequence
QVWDSSAYV

SEQ ID NO: 104 - protein, 274 aa, Artificial Sequence
MPIWKFPDEEGACQPCPINCTHSCVDLDDKGCPAEQRASPLTEPKSSDKTHTCPPCPAPELLGGPSVFLFPPKPKDTLMISRTPEVTCVVVDVSHEDPEVKFNWYVDGVEVHNAKTKPREEQYNSTYRVVSVLTVLHQDWLNGKEYKCKVSNKALPAPIEKTISKAKGQPREPQVYTLPPSREEMTKNQVSLTCLVKGFYPSDIAVEWESNGQPENNYKTTPPVLDSDGSFFLYSKLTVDKSRWQQGNVFSCSVMHEALHNHYTQKSLSLSPGK

SEQ ID NO: 105 - protein, 377 aa, homo sapiens
QETELSVSAELVPTSSWNISSELNKDSYLTLDEPMNNITTSLGQTAELHCKVSGNPPPTIRWFKNDAPVVQEPRRLSFRSTIYGSRLRIRNLDTTDTGYFQCVATNGKEVVSSTGVLFVKFGPPPTASPGYSDEYEEDGFCQPYRGIACARFIGNRTVYMESLHMQGEIENQITAAFTMIGTSSHLSDKCSQFAIPSLCHYAFPYCDETSSVPKPRDLCRDECEILENVLCQTEYIFARSNPMILMRLKLPNCEDLPQPESPEAANCIRIGIPMADPINKNHKCYNSTGVDYRGTVSVTKSGRQCQPWNSQYPHTHTFTALRFPELNGGHSYCRNPGNQKEAPWCFTLDENFKSDLCDIPACDSKDSKEKNKMEILY